European Patent Application EP 4 173 617 A1, published May 3, 2023. Title: IRON OXIDE NANOPARTICLES WITH ANTIVIRAL ACTIVITY AGAINST SARS AND MERS         CORONAVIRUS. Applicant: CONSEJO SUPERIOR DE INVESTIGACIONES CIENTÍFICAS (CSIC). The sequence listing filed with the application follows.

SEQUENCE LISTING (6 sequences)

SEQ ID NO: 1 - DNA, 22 bp, Artificial sequence
  qPCR Primer SARS-2-RdRp-15431-VS
gtgaaatggtcatgtgtggcgg

SEQ ID NO: 2 - DNA, 26 bp, Artificial Sequence
  qPCR primer SARS-2-RdRp-15530-RS
caaatgttaaaaacactattagcata

SEQ ID NO: 3 - DNA, 24 bp, Artificial sequence
  NPs primer SARS-2-leader-VS
tcccaggtaacaaaccaaccaact

SEQ ID NO: 4 - DNA, 20 bp, Artificial Sequence
  Primer SARS-2-7a-RS
aaatggtgaattgccctcgt

SEQ ID NO: 5 - DNA, 24 bp, Artificial Sequence
  GAPDH primer 1
tgccatgggtggaatcatattgga

SEQ ID NO: 6 - DNA, 24 bp, Artificial sequence
  GAPDH primer 2
tcggagtcaacggatttgggtcgt